European Patent Specification EP 3 287 470 B1, published July 12, 2023. Title: NOVEL RECOMBINANT BI-FUNCTIONAL FUSION PROTEIN AND PREPARATION AND APPLICATION THEREFOR. Applicant: Immuneonco Biopharmaceuticals (Shanghai) Co., Ltd. Application 15889744.7. The sequence listing filed with the application follows.

SEQUENCE LISTING (13 sequences)

SEQ ID NO: 1 - DNA, 1752 bp, Homo sapiens
tcctgcgcctggtcaggagtggcgggtgaggaggagctgcaggtgattcagcctgacaagtccgtatcagttgcagctggagagtcggccattctgcactgcactgtgacctccctgatccctgtggggcccatccagtggttcagaggagctggaccagcccgggaattaatctacaatcaaaaagaaggccacttcccccgggtaacaactgtttcagagtccacaaagagagaaaacatggacttttccatcagcatcagtaacatcaccccagcagatgccggcacctactactgtgtgaagttccggaaagggagccctgacacggagtttaagtctggagcaggcactgagctgtctgtgcgtgccaaaccctctgcccccgtggtatcgggccctgcggcgagggccacacctcagcacacagtgagcttcacctgcgagtcccacggcttctcacccagagacatcaccctgaaatggttcaaaaatgggaatgagctctcagacttccagaccaacgtggaccccgtaggagagagcgtgtcctacagcatccacagcacagccaaggtggtgctgacccgcgaggacgttcactctcaagtcatctgcgaggtggcccacgtcaccttgcagggggaccctcttcgtgggactgccaacttgtctgagaccatccgagttccacccaccttggaggttactcaacagcccgtgagggcagagaaccaggtgaatgtcacctgccaggtgaggaagttctacccccagagactacagctgacctggttggagaatggaaacgtgtcccggacagaaacggcctcaaccgttacagagaacaaggatggtacctacaactggatgagctggctcctggtgaatgtatctgcccacagggatgatgtgaagctcacctgccaggtggagcatgacgggcagccagcggtcagcaaaagccatgacctgaaggtctcagcccacccgaaggagcagggctcaaataccgccgctgagaacactggatctaatgaacggaacgaattcgagcccaaatcttgtgacaaaactcacacatgcccaccgtgcccagcacctgaactcctggggggaccgtcagtcttcctcttccccccaaaacccaaggacaccctcatgatctcccggacccctgaggtcacatgcgtggtggtggacgtgagccacgaagaccctgaggtcaagttcaactggtacgtggacggcgtggaggtgcataatgccaagacaaagccgcgggaggagcagtacaacagcacgtaccgtgtggtcagcgtcctcaccgtcctgcaccaggactggctgaatggcaaggagtacaagtgcaaggtctccaacaaagccctcccagcccccatcgagaaaaccatctccaaagccaaagggcagccccgagaaccacaggtgtacaccctgcccccatcccgggatgagctgaccaagaaccaggtcagcctgacctgcctggtcaaaggcttctatcccagcgacatcgccgtggagtgggagagcaatgggcagccggagaacaactacaagaccacgcctcccgtgctggactccgacggctccttcttcctctacagcaagctcaccgtggacaagagcaggtggcagcaggggaacgtcttctcatgctccgtgatgcatgaggctctgcacaaccactacacgcagaagagcctctccctgtctccgggtaaatga

SEQ ID NO: 2 - protein, 583 aa, Homo sapiens
SCAWSGVAGEEELQVIQPDKSVSVAAGESAILHCTVTSLIPVGPIQWFRGAGPARELIYNQKEGHFPRVTTVSESTKRENMDFSISISNITPADAGTYYCVKFRKGSPDTEFKSGAGTELSVRAKPSAPVVSGPAARATPQHTVSFTCESHGFSPRDITLKWFKNGNELSDFQTNVDPVGESVSYSIHSTAKVVLTREDVHSQVICEVAHVTLQGDPLRGTANLSETIRVPPTLEVTQQPVRAENQVNVTCQVRKFYPQRLQLTWLENGNVSRTETASTVTENKDGTYNWMSWLLVNVSAHRDDVKLTCQVEHDGQPAVSKSHDLKVSAHPKEQGSNTAAENTGSNERNEFEPKSCDKTHTCPPCPAPELLGGPSVFLFPPKPKDTLMISRTPEVTCVVVDVSHEDPEVKFNWYVDGVEVHNAKTKPREEQYNSTYRVVSVLTVLHQDWLNGKEYKCKVSNKALPAPIEKTISKAKGQPREPQVYTLPPSRDELTKNQVSLTCLVKGFYPSDIAVEWESNGQPENNYKTTPPVLDSDGSFFLYSKLTVDKSRWQQGNVFSCSVMHEALHNHYTQKSLSLSPGK

SEQ ID NO: 3 - DNA, 1131 bp, Homo sapiens
tcctgcgcctggtcaggagtggcgggtgaggaggagctgcaggtgattcagcctgacaagtccgtatcagttgcagctggagagtcggccattctgcactgcactgtgacctccctgatccctgtggggcccatccagtggttcagaggagctggaccagcccgggaattaatctacaatcaaaaagaaggccacttcccccgggtaacaactgtttcagagtccacaaagagagaaaacatggacttttccatcagcatcagtaacatcaccccagcagatgccggcacctactactgtgtgaagttccggaaagggagccctgacacggagtttaagtctggagcaggcactgagctgtctgtgcgtgccaaaccctctgcccccgtggtatcgggccctgcggcgagggccacacctcagcacgaattcgagcccaaatcttgtgacaaaactcacacatgcccaccgtgcccagcacctgaactcctggggggaccgtcagtcttcctcttccccccaaaacccaaggacaccctcatgatctcccggacccctgaggtcacatgcgtggtggtggacgtgagccacgaagaccctgaggtcaagttcaactggtacgtggacggcgtggaggtgcataatgccaagacaaagccgcgggaggagcagtacaacagcacgtaccgtgtggtcagcgtcctcaccgtcctgcaccaggactggctgaatggcaaggagtacaagtgcaaggtctccaacaaagccctcccagcccccatcgagaaaaccatctccaaagccaaagggcagccccgagaaccacaggtgtacaccctgcccccatcccgggatgagctgaccaagaaccaggtcagcctgacctgcctggtcaaaggcttctatcccagcgacatcgccgtggagtgggagagcaatgggcagccggagaacaactacaagaccacgcctcccgtgctggactccgacggctccttcttcctctacagcaagctcaccgtggacaagagcaggtggcagcaggggaacgtcttctcatgctccgtgatgcatgaggctctgcacaaccactacacgcagaagagcctctccctgtctccgggtaaatag

SEQ ID NO: 4 - protein, 376 aa, Homo sapiens
SCAWSGVAGEEELQVIQPDKSVSVAAGESAILHCTVTSLIPVGPIQWFRGAGPARELIYNQKEGHFPRVTTVSESTKRENMDFSISISNITPADAGTYYCVKFRKGSPDTEFKSGAGTELSVRAKPSAPVVSGPAARATPQHEFEPKSCDKTHTCPPCPAPELLGGPSVFLFPPKPKDTLMISRTPEVTCVVVDVSHEDPEVKFNWYVDGVEVHNAKTKPREEQYNSTYRVVSVLTVLHQDWLNGKEYKCKVSNKALPAPIEKTISKAKGQPREPQVYTLPPSRDELTKNQVSLTCLVKGFYPSDIAVEWESNGQPENNYKTTPPVLDSDGSFFLYSKLTVDKSRWQQGNVFSCSVMHEALHNHYTQKSLSLSPGK

SEQ ID NO: 5 - DNA, 1125 bp, Homo sapiens
tcctgcgcctggtcaggagtggcgggtgaggaggagctgcaggtgattcagcctgacaagtccgtatcagttgcagctggagagtcggccattctgcactgcactgtgacctccctgatccctgtggggcccatccagtggttcagaggagctggaccagcccgggaattaatctacaatcaaaaagaaggccacttcccccgggtaacaactgtttcagagtccacaaagagagaaaacatggacttttccatcagcatcagtgccatcaccccagcagatgccggcacctactactgtgtgaagttccggaaagggagccctgacacggagtttaagtctggagcaggcactgagctgtctgtgcgtgccaaaccctctgcccccgtggtatcgggccctgcggcgagggccacacctcagcacgagcccaaatcttgtgacaaaactcacacatgcccaccgtgcccagcacctgaactcctggggggaccgtcagtcttcctcttccccccaaaacccaaggacaccctcatgatctcccggacccctgaggtcacatgcgtggtggtggacgtgagccacgaagaccctgaggtcaagttcaactggtacgtggacggcgtggaggtgcataatgccaagacaaagccgcgggaggagcagtacaacagcacgtaccgtgtggtcagcgtcctcaccgtcctgcaccaggactggctgaatggcaaggagtacaagtgcaaggtctccaacaaagccctcccagcccccatcgagaaaaccatctccaaagccaaagggcagccccgagaaccacaggtgtacaccctgcccccatcccgggatgagctgaccaagaaccaggtcagcctgacctgcctggtcaaaggcttctatcccagcgacatcgccgtggagtgggagagcaatgggcagccggagaacaactacaagaccacgcctcccgtgctggactccgacggctccttcttcctctacagcaagctcaccgtggacaagagcaggtggcagcaggggaacgtcttctcatgctccgtgatgcatgaggctctgcacaaccactacacgcagaagagcctctccctgtctccgggtaaatag

SEQ ID NO: 6 - protein, 374 aa, Homo sapiens
SCAWSGVAGEEELQVIQPDKSVSVAAGESAILHCTVTSLIPVGPIQWFRGAGPARELIYNQKEGHFPRVTTVSESTKRENMDFSISISAITPADAGTYYCVKFRKGSPDTEFKSGAGTELSVRAKPSAPVVSGPAARATPQHEPKSCDKTHTCPPCPAPELLGGPSVFLFPPKPKDTLMISRTPEVTCVVVDVSHEDPEVKFNWYVDGVEVHNAKTKPREEQYNSTYRVVSVLTVLHQDWLNGKEYKCKVSNKALPAPIEKTISKAKGQPREPQVYTLPPSRDELTKNQVSLTCLVKGFYPSDIAVEWESNGQPENNYKTTPPVLDSDGSFFLYSKLTVDKSRWQQGNVFSCSVMHEALHNHYTQKSLSLSPGK

SEQ ID NO: 7 - DNA, 1125 bp, Homo sapiens
tcctgcgcctggtcaggagtggcgggtgaggaggagctgcaggtgattcagcctgacaagtccgtatcagttgcagctggagagtcggccattctgcactgcactgtgacctccctgatccctgtggggcccatccagtggttcagaggagctggaccagcccgggaattaatctacaatcaaaaagaaggccacttcccccgggtaacaactgtttcagagtccacaaagagagaaaacatggacttttccatcagcatcagtgccatcaccccagcagatgccggcacctactactgtgtgaagttccggaaagggagccctgacacggagtttaagtctggagcaggcactgagctgtctgtgcgtgccaaaccctctgcccccgtggtatcgggccctgcggcgagggccacacctcagcacgagcccaaatcttgtgacaaaactcacacatgcccaccgtgcccagcacctgaactcctggggggaccgtcagtcttcctcttccccccaaaacccaaggacaccctcatgatctcccggacccctgaggtcacatgcgtggtggtggccgtgagccacgaagaccctgaggtcaagttcaactggtacgtggacggcgtggaggtgcataatgccaagacaaagccgcgggaggagcagtacaacagcacgtaccgtgtggtcagcgtcctcaccgtcctgcaccaggactggctgaatggcaaggagtacaagtgcaaggtctccaacaaagccctcccagcccccatcgagaaaaccatctccaaagccaaagggcagccccgagaaccacaggtgtacaccctgcccccatcccgggatgagctgaccaagaaccaggtcagcctgacctgcctggtcaaaggcttctatcccagcgacatcgccgtggagtgggagagcaatgggcagccggagaacaactacaagaccacgcctcccgtgctggactccgacggctccttcttcctctacagcaagctcaccgtggacaagagcaggtggcagcaggggaacgtcttctcatgctccgtgatgcatgaggctctgcacaaccactacacgcagaagagcctctccctgtctccgggtaaatag

SEQ ID NO: 8 - protein, 374 aa, Homo sapiens
SCAWSGVAGEEELQVIQPDKSVSVAAGESAILHCTVTSLIPVGPIQWFRGAGPARELIYNQKEGHFPRVTTVSESTKRENMDFSISISAITPADAGTYYCVKFRKGSPDTEFKSGAGTELSVRAKPSAPVVSGPAARATPQHEPKSCDKTHTCPPCPAPELLGGPSVFLFPPKPKDTLMISRTPEVTCVVVAVSHEDPEVKFNWYVDGVEVHNAKTKPREEQYNSTYRVVSVLTVLHQDWLNGKEYKCKVSNKALPAPIEKTISKAKGQPREPQVYTLPPSRDELTKNQVSLTCLVKGFYPSDIAVEWESNGQPENNYKTTPPVLDSDGSFFLYSKLTVDKSRWQQGNVFSCSVMHEALHNHYTQKSLSLSPGK

SEQ ID NO: 9 - DNA, 40 bp, Artificial sequence
  Primer
cccaagcttggggccaccatggagcccgccggcccggccc

SEQ ID NO: 10 - DNA, 30 bp, Artificial sequence
  Primer
cggaattcgttccgttcattagatccagtg

SEQ ID NO: 11 - DNA, 30 bp, Artificial sequence
  Primer
cggaattcgtgctgaggtgtggccctcgcc

SEQ ID NO: 12 - DNA, 43 bp, Artificial sequence
  Primer
gaggtcacatgcgtggtggtggccgtgagccacgaagaccctg

SEQ ID NO: 13 - DNA, 40 bp, Artificial sequence
  Primer
caccaccacgcatgtgacctcaggggtccgggagatcatg